European Patent Specification EP 4 121 117 B1, published October 8, 2025. Title: DESIGNER EXTRACELLULAR VESICLES FOR TREATING EXCITOTOXICITY. Applicant: Ohio State Innovation Foundation. The sequence listing filed with the application follows.

SEQUENCE LISTING (14 sequences)

SEQ ID NO: 1 - DNA, 2496 bp, Mus musculus
atgtccgggaagggaggctgggcctggtggtgggcccggctgcccctctgcctactcctcagcctttatggctcctgggtgccttcatccctaggaaagcccaagggtcacccccacatgaactctatccgtatcgatggagacatcaccctgggaggcctgtttcccgtccacggtcgcggctccgagggcaaggcctgcggcgagttgaagaaggagaaaggtatccaccggctggaggccatgctctttgccctggaccgcatcaacaacgacccggacctactgcccaacatcacgttgggcgcccgcattctggacacctgctcaagggatacccacgccctggagcagtccctgacctttgtgcaggcgctcatcgagaaggacggcacggaggtccgctgcggcagcgggggcccacccatcatcaccaagcctgaacgagtggtgggtgtcatcggagcttcggggagctccgtctcgatcatggtggccaacatcctccgcctcttcaagatcccccagatcagctacgcctccacggctcccgacttgagtgataacagccgctatgacttcttctcccgggtcgtgccctcggacacataccaggcccaggccatggtggacatcgtccgggccctcaagtggaactatgtgtccacgctggcctcagagggtagctacggcgagagcggcgtggaggcctttatccagaagtcccgagagaacggaggcgtgtgcattgcccagtcggtgaagattccacgggaacccaagaccggggagtttgacaagatcatcaaacgccttctggaaacgtccaatgccagagccatcatcatctttgccaacgaggatgatatcaggagggtgctggaggcagcgcgcagggccaaccagaccggccacttcttttggatgggttctgatagctggggctccaagagcgcccccgtgctgcgccttgaggaagtggctgaaggtgcagtcaccattcttcccaagaggacgtctgtgcgagggtttgaccgatacttctccagccgcacgcttgacaacaacaggcgcaacatctggtttgctgagttctgggaggacaacttccattgcaagttgagccgccacgcgctcaagaagggaagccacatcaagaagtgcaccaaccgagagcgcatcgggcaggactcggcctacgaacaggaggggaaggtgcagtttgtgatcgacgccgtgtacgccatgggccatgctctgcacgccatgcatcgtgacctgtgtcccggccgcgtaggactctgccctcgaatggaccctgtggatggcacccagctgcttaagtacatcagaaacgtcaacttctcaggcatcgccgggaacccggtgaccttcaacgagaacggagacgcgccagggcgttatgacatctaccagtaccaacgtcgcaacggctcggctgagtacaaggtcatcggctcatggacagaccacttgcacctcagaatagagcggatgcagtggccagggagtggccagcagctgccacgctccatctgcagcctgccctgccagccaggcgagcggaagaagacggtgaagggcatggcttgctgctggcactgcgagccctgcacggggtaccagtaccaggtggaccgctacacctgtaagacctgcccctatgacatgcggcccacggagaaccgcacgagctgccagcccatacccattgtcaagttggagtgggactcaccctgggctgtgctgcccctcttcctggctgtggtgggcattgctgccacgctgttcgtggtggtcacttttgtgcgctacaacgacactccgatcgtcaaggcctcgggccgggagctgagctacgtcctgctggcgggcatctttctctgctatgccaccaccttcctcatgatcgcagagcctgacctggggacctgttcactccgccgcatcttcctggggcttggcatgagcatcagctacgcggccctgctgaccaagaccaaccgcatctaccgcatctttgagcagggcaagcggtcggtcagcgccccacggttcatcagccccgcctcgcagctggccatcaccttcgtcctcatctcgctgcagttgcttggcatctgcgtgtggttcgtggtggacccctcccactcggtggtggacttccaggaccagcggacacttgacccccgcttcgcccggggtgtgctcaagtgtgacatctcggacctgtcgctcatctgcctcctgggctacagcatgctgctgatggtcacgtgtactgtgtatgccatcaagactcgaggcgtgcctgagaccttcaatgaggccaagcccatcggcttcaccatgtacaccacctgcatcgtctggctggccttcatccccatcttttttggcacctcgcagtcggctgacaaggtaacctctgaggccctgcccgtggaattcagcccgccattgctggcacataat

SEQ ID NO: 2 - protein, 832 aa, Mus musculus
MSGKGGWAWWWARLPLCLLLSLYGSWVPSSLGKPKGHPHMNSIRIDGDITLGGLFPVHGRGSEGKACGELKKEKGIHRLEAMLFALDRINNDPDLLPNITLGARILDTCSRDTHALEQSLTFVQALIEKDGTEVRCGSGGPPIITKPERVVGVIGASGSSVSIMVANILRLFKIPQISYASTAPDLSDNSRYDFFSRVVPSDTYQAQAMVDIVRALKWNYVSTLASEGSYGESGVEAFIQKSRENGGVCIAQSVKIPREPKTGEFDKIIKRLLETSNARAIIIFANEDDIRRVLEAARRANQTGHFFWMGSDSWGSKSAPVLRLEEVAEGAVTILPKRTSVRGFDRYFSSRTLDNNRRNIWFAEFWEDNFHCKLSRHALKKGSHIKKCTNRERIGQDSAYEQEGKVQFVIDAVYAMGHALHAMHRDLCPGRVGLCPRMDPVDGTQLLKYIRNVNFSGIAGNPVTFNENGDAPGRYDIYQYQRRNGSAEYKVIGSWTDHLHLRIERMQWPGSGQQLPRSICSLPCQPGERKKTVKGMACCWHCEPCTGYQYQVDRYTCKTCPYDMRPTENRTSCQPIPIVKLEWDSPWAVLPLFLAVVGIAATLFVVVTFVRYNDTPIVKASGRELSYVLLAGIFLCYATTFLMIAEPDLGTCSLRRIFLGLGMSISYAALLTKTNRIYRIFEQGKRSVSAPRFISPASQLAITFVLISLQLLGICVWFVVDPSHSVVDFQDQRTLDPRFARGVLKCDISDLSLICLLGYSMLLMVTCTVYAIKTRGVPETFNEAKPIGFTMYTTCIVWLAFIPIFFGTSQSADKVTSEALPVEFSPPLLAHN

SEQ ID NO: 3 - DNA, 2724 bp, Mus musculus
atggtttgtgagggaaagcgctcaacctcttgcccttgtttcttccttttgactgccaagttctactggatcctcacaatgatgcaaagaactcacagccaggagtatgcgcattccatccgcctggatggggacatcattttggggggtctttttcctgttcatgccaagggagaaagaggggtgccttgtggggacctgaagaaggaaaagggcatccacagacttgaggccatgctttatgcaatcgaccagattaataaggaccccgatctcctctccaatatcactctgggtgtccggatccttgacacatgttccagggacacctatgctttggagcagtcactaaccttcgtgcaggcactgatagagaaagacgcgtctgacgtgaagtgtgctaatggagacccacccatattcaccaagcccgacaagatttctggtgtcataggtgctgcagcaagctccgtgtccatcatggtggctaacattttaagactttttaagatacctcagattagctatgcatctacagccccagagctaagtgacaacaccaggtatgatttcttttctcgggtggtcccgcctgactcctaccaagcccaagccatggtggacattgtgacagccctgggatggaattatgtgtcaacactggcttccgaggggaactatggagagagtggtgttgaggccttcactcagatctcaagggagattggtggtgtttgcattgctcaatcacagaaaatcccacgtgaaccaagacctggagaattcgaaaaaattatcaaacgcctgctggagacacccaacgctcgcgcagtgattatgtttgccaatgaggatgacatcaggaggatattggaagcagcaaaaaaattaaaccagagtgggcattttctatggattggctcagatagttggggatccaaaatagcacctgtctatcagcaggaggagatcgccgaaggagctgtgacaattttgcccaaaagagcatcaattgatgggtttgaccgatactttagaagccgaactcttgccaataatcgaagaaatgtgtggtttgcagaattttgggaggagaattttggatgcaaattaggatcacatgggaagaggaacagtcatataaagaaatgcacagggctggagcgaattgcacgggattcatcttacgaacaagaaggaaaggttcaatttgtaattgatgcagtgtattccatggcttatgcactgcacaacatgcacaaagaactctgccctggttacataggcctttgcccaaggatggttaccatcgatgggaaagagctactgggttacatcagggccgtgaattttaatggcagcgctggtacacctgtcacttttaatgagaatggagatgctccgggacgctacgatatcttccaatatcagataaacaacaaaagtacagaatacaaaatcatcggccactggaccaatcaacttcacctaaaagtggaagacatgcagtgggctaatagagagcacacgcacccagcatctgtctgcagcctgccgtgcaagcctggggagaggaagaaaaccgtgaaaggggtcccttgctgctggcactgtgaacgctgcgagggttataactaccaggtggacgaactctcctgtgaactctgccctttggatcagagaccaaacatcaaccgcactggctgccagaggattcccatcatcaagttggagtggcattcaccctgggccgtggtacctgtgttcatagcaatattgggaatcattgccaccacctttgtgattgtgacctttgtccgctataatgacacaccaatcgtgagagcttctgggcgggaacttagttatgtgctcctaacggggatttttctctgttactcaatcacttttttgatgattgcggcacctgacacaatcatctgctctttccgaaggatcttcctgggacttggtatgtgtttcagctatgcagcacttttgaccaaaacaaaccgtatccaccgaatattcgagcaagggaagaaatctgtcacagcacctaagttcatcagcccagcatcccagctggtgatcaccttcagcctcatctccgtacagctccttggagtgtttgtgtggtttgtcgtggatcccccccacaccatcattgactatggagaacagcgaacactggatcccgagaacgccaggggagtgctcaagtgtgacatttccgatctgtcactcatttgttcactgggatacagtatcctcctgatggtcacttgtactgtttatgccattaaaaccagaggggttccagaaacgttcaatgaagccaaacctattggatttaccatgtacaccacgtgcatcatttggttagctttcattcccatcttttttggtacagcccagtcagcagaaaagatgtacatccagacaacaacacttactgtctccatgagtttaagtgcttcagtgtctctgggaatgctctatatgcccaaagtttatattataatttttcatccagagcagaacgttcaaaaacgcaagagaagcttcaaggctgtggtcacggccgctaccatgcaaagcaaactgatccaaaagggaaatgacagaccaaacggcgaggtgaaaagtgaactctgtgagagtcttgaaaccaacagtaagtcatctgtagactttcagatggtcaagagcgggagcacttcc

SEQ ID NO: 4 - protein, 908 aa, Mus musculus
MVCEGKRSTSCPCFFLLTAKFYWILTMMQRTHSQEYAHSIRLDGDIILGGLFPVHAKGERGVPCGDLKKEKGIHRLEAMLYAIDQINKDPDLLSNITLGVRILDTCSRDTYALEQSLTFVQALIEKDASDVKCANGDPPIFTKPDKISGVIGAAASSVSIMVANILRLFKIPQISYASTAPELSDNTRYDFFSRVVPPDSYQAQAMVDIVTALGWNYVSTLASEGNYGESGVEAFTQISREIGGVCIAQSQKIPREPRPGEFEKIIKRLLETPNARAVIMFANEDDIRRILEAAKKLNQSGHFLWIGSDSWGSKIAPVYQQEEIAEGAVTILPKRASIDGFDRYFRSRTLANNRRNVWFAEFWEENFGCKLGSHGKRNSHIKKCTGLERIARDSSYEQEGKVQFVIDAVYSMAYALHNMHKELCPGYIGLCPRMVTIDGKELLGYIRAVNFNGSAGTPVTFNENGDAPGRYDIFQYQINNKSTEYKIIGHWTNQLHLKVEDMQWANREHTHPASVCSLPCKPGERKKTVKGVPCCWHCERCEGYNYQVDELSCELCPLDQRPNINRTGCQRIPIIKLEWHSPWAVVPVFIAILGIIATTFVIVTFVRYNDTPIVRASGRELSYVLLTGIFLCYSITFLMIAAPDTIICSFRRIFLGLGMCFSYAALLTKTNRIHRIFEQGKKSVTAPKFISPASQLVITFSLISVQLLGVFVWFVVDPPHTIIDYGEQRTLDPENARGVLKCDISDLSLICSLGYSILLMVTCTVYAIKTRGVPETFNEAKPIGFTMYTTCIIWLAFIPIFFGTAQSAEKMYIQTTTLTVSMSLSASVSLGMLYMPKVYIIIFHPEQNVQKRKRSFKAVVTAATMQSKLIQKGNDRPNGEVKSELCESLETNSKSSVDFQMVKSGSTS

SEQ ID NO: 5 - DNA, 2736 bp, Homo sapiens
atgcctgggaagagaggcttgggctggtggtgggcccggctgcccctttgcctgctcctcagcctttacggcccctggatgccttcctccctgggaaagcccaaaggccaccctcacatgaattccatccgcatagatggggacatcacactgggaggcctgttcccggtgcatggccggggctcagagggcaagccctgtggagaacttaagaaggaaaagggcatccaccggctggaggccatgctgttcgccctggatcgcatcaacaacgacccggacctgctgcctaacatcacgctgggcgcccgcattctggacacctgctccagggacacccatgccctcgagcagtcgctgacctttgtgcaggcgctcatcgagaaggatggcacagaggtccgctgtggcagtggcggcccacccatcatcaccaagcctgaacgtgtggtgggtgtcatcggtgcttcagggagctcggtctccatcatggtggccaacatccttcgcctcttcaagataccccagatcagctacgcctccacagcgccagacctgagtgacaacagccgctacgatttcttctcccgcgtggtgccctcggacacgtaccaggcccaggccatggtggacatcgtccgtgccctcaagtggaactatgtgtccacagtggcctcggagggcagctatggtgagagcggtgtggaggccttcatccagaagtcccgtgaggacgggggcgtgtgcatcgcccagtcggtgaagataccacgggagcccaaggcaggcgagttcgacaagatcatccgccgcctcctggagacttcgaacgccagggcagtcatcatctttgccaacgaggatgacatcaggcgtgtgctggaggcagcacgaagggccaaccagacaggccatttcttctggatgggctctgacagctggggctccaagattgcacctgtgctgcacctggaggaggtggctgagggtgctgtcacgatcctccccaagaggatgtccgtacgaggcttcgaccgctacttctccagccgcacgctggacaacaaccggcgcaacatctggtttgccgagttctgggaggacaacttccactgcaagctgagccgccacgccctcaagaagggcagccacgtcaagaagtgcaccaaccgtgagcgaattgggcaggattcagcttatgagcaggaggggaaggtgcagtttgtgatcgatgccgtgtacgccatgggccacgcgctgcacgccatgcaccgtgacctgtgtcccggccgcgtggggctctgcccgcgcatggaccctgtagatggcacccagctgcttaagtacatccgaaacgtcaacttctcaggcatcgcagggaaccctgtgaccttcaatgagaatggagatgcgcctgggcgctatgacatctaccaataccagctgcgcaacgattctgccgagtacaaggtcattggctcctggactgaccacctgcaccttagaatagagcggatgcactggccggggagcgggcagcagctgccccgctccatctgcagcctgccctgccaaccgggtgagcggaagaagacagtgaagggcatgccttgctgctggcactgcgagccttgcacagggtaccagtaccaggtggaccgctacacctgtaagacgtgtccctatgacatgcggcccacagagaaccgcacgggctgccggcccatccccatcatcaagcttgagtggggctcgccctgggccgtgctgcccctcttcctggccgtggtgggcatcgctgccacgttgttcgtggtgatcacctttgtgcgctacaacgacacgcccatcgtcaaggcctcgggccgtgaactgagctacgtgctgctggcaggcatcttcctgtgctatgccaccaccttcctcatgatcgctgagcccgaccttggcacctgctcgctgcgccgaatcttcctgggactagggatgagcatcagctatgcagccctgctcaccaagaccaaccgcatctaccgcatcttcgagcagggcaagcgctcggtcagtgccccacgcttcatcagccccgcctcacagctggccatcaccttcagcctcatctcgctgcagctgctgggcatctgtgtgtggtttgtggtggacccctcccactcggtggtggacttccaggaccagcggacactcgacccccgcttcgccaggggtgtgctcaagtgtgacatctcggacctgtcgctcatctgcctgctgggctacagcatgctgctcatggtcacgtgcaccgtgtatgccatcaagacacgcggcgtgcccgagaccttcaatgaggccaagcccattggcttcaccatgtacaccacttgcatcgtctggctggccttcatccccatcttctttggcacctcgcagtcggccgacaagctgtacatccagacgacgacgctgacggtctcggtgagtctgagcgcctcggtgtccctgggaatgctctacatgcccaaagtctacatcatcctcttccacccggagcagaatgtgcccaagcgcaagcgcagcctcaaagccgtcgttacggcggccaccatgtccaacaagttcacgcagaagggcaacttccggcccaacggagaggccaagtctgagctctgcgagaaccttgaggccccagcgctggccaccaaacagacttacgtcacttacaccaaccatgcaatc

SEQ ID NO: 6 - protein, 912 aa, Homo sapiens
MPGKRGLGWWWARLPLCLLLSLYGPWMPSSLGKPKGHPHMNSIRIDGDITLGGLFPVHGRGSEGKPCGELKKEKGIHRLEAMLFALDRINNDPDLLPNITLGARILDTCSRDTHALEQSLTFVQALIEKDGTEVRCGSGGPPIITKPERVVGVIGASGSSVSIMVANILRLFKIPQISYASTAPDLSDNSRYDFFSRVVPSDTYQAQAMVDIVRALKWNYVSTVASEGSYGESGVEAFIQKSREDGGVCIAQSVKIPREPKAGEFDKIIRRLLETSNARAVIIFANEDDIRRVLEAARRANQTGHFFWMGSDSWGSKIAPVLHLEEVAEGAVTILPKRMSVRGFDRYFSSRTLDNNRRNIWFAEFWEDNFHCKLSRHALKKGSHVKKCTNRERIGQDSAYEQEGKVQFVIDAVYAMGHALHAMHRDLCPGRVGLCPRMDPVDGTQLLKYIRNVNFSGIAGNPVTFNENGDAPGRYDIYQYQLRNDSAEYKVIGSWTDHLHLRIERMHWPGSGQQLPRSICSLPCQPGERKKTVKGMPCCWHCEPCTGYQYQVDRYTCKTCPYDMRPTENRTGCRPIPIIKLEWGSPWAVLPLFLAVVGIAATLFVVITFVRYNDTPIVKASGRELSYVLLAGIFLCYATTFLMIAEPDLGTCSLRRIFLGLGMSISYAALLTKTNRIYRIFEQGKRSVSAPRFISPASQLAITFSLISLQLLGICVWFVVDPSHSVVDFQDQRTLDPRFARGVLKCDISDLSLICLLGYSMLLMVTCTVYAIKTRGVPETFNEAKPIGFTMYTTCIVWLAFIPIFFGTSQSADKLYIQTTTLTVSVSLSASVSLGMLYMPKVYIILFHPEQNVPKRKRSLKAVVTAATMSNKFTQKGNFRPNGEAKSELCENLEAPALATKQTYVTYTNHAI

SEQ ID NO: 7 - DNA, 2724 bp, Homo sapiens
atggtatgcgagggaaagcgatcagcctcttgcccttgtttcttcctcttgaccgccaagttctactggatcctcacaatgatgcaaagaactcacagccaggagtatgcccattccatacgggtggatggggacattattttggggggtctcttccctgtccacgcaaagggagagagaggggtgccttgtggggagctgaagaaggaaaaggggattcacagactggaggccatgctttatgcaattgaccagattaacaaggaccctgatctcctttccaacatcactctgggtgtccgcatcctcgacacgtgctctagggacacctatgctttggagcagtctctaacattcgtgcaggcattaatagagaaagatgcttcggatgtgaagtgtgctaatggagatccacccattttcaccaagcccgacaagatttctggcgtcataggtgctgcagcaagctccgtgtccatcatggttgctaacattttaagactttttaagatacctcaaatcagctatgcatccacagccccagagctaagtgataacaccaggtatgactttttctctcgagtggttccgcctgactcctaccaagcccaagccatggtggacatcgtgacagcactgggatggaattatgtttcgacactggcttctgaggggaactatggtgagagcggtgtggaggccttcacccagatctcgagggagattggtggtgtttgcattgctcagtcacagaaaatcccacgtgaaccaagacctggagaatttgaaaaaattatcaaacgcctgctagaaacacctaatgctcgagcagtgattatgtttgccaatgaggatgacatcaggaggatattggaagcagcaaaaaaactaaaccaaagtgggcattttctctggattggctcagatagttggggatccaaaatagcacctgtctatcagcaagaggagattgcagaaggggctgtgacaattttgcccaaacgagcatcaattgatggatttgatcgatactttagaagccgaactcttgccaataatcgaagaaatgtgtggtttgcagaattctgggaggagaattttggctgcaagttaggatcacatgggaaaaggaacagtcatataaagaaatgcacagggctggagcgaattgctcgggattcatcttatgaacaggaaggaaaggtccaatttgtaattgatgctgtatattccatggcttacgccctgcacaatatgcacaaagatctctgccctggatacattggcctttgtccacgaatgagtaccattgatgggaaagagctacttggttatattcgggctgtaaattttaatggcagtgctggcactcctgtcacttttaatgaaaacggagatgctcctggacgttatgatatcttccagtatcaaataaccaacaaaagcacagagtacaaagtcatcggccactggaccaatcagcttcatctaaaagtggaagacatgcagtgggctcatagagaacatactcacccggcgtctgtctgcagcctgccgtgtaagccaggggagaggaagaaaacggtgaaaggggtcccttgctgctggcactgtgaacgctgtgaaggttacaactaccaggtggatgagctgtcctgtgaactttgccctctggatcagagacccaacatgaaccgcacaggctgccagcttatccccatcatcaaattggagtggcattctccctgggctgtggtgcctgtgtttgttgcaatattgggaatcatcgccaccacctttgtgatcgtgacctttgtccgctataatgacacacctatcgtgagggcttcaggacgcgaacttagttacgtgctcctaacggggatttttctctgttattcaatcacgtttttaatgattgcagcaccagatacaatcatatgctccttccgacgggtcttcctaggacttggcatgtgtttcagctatgcagcccttctgaccaaaacaaaccgtatccaccgaatatttgagcaggggaagaaatctgtcacagcgcccaagttcattagtccagcatctcagctggtgatcaccttcagcctcatctccgtccagctccttggagtgtttgtctggtttgttgtggatcccccccacatcatcattgactatggagagcagcggacactagatccagagaaggccaggggagtgctcaagtgtgacatttctgatctctcactcatttgttcacttggatacagtatcctcttgatggtcacttgtactgtttatgccattaaaacgagaggtgtcccagagactttcaatgaagccaaacctattggatttaccatgtataccacctgcatcatttggttagctttcatccccatcttttttggtacagcccagtcagcagaaaagatgtacatccagacaacaacacttactgtctccatgagtttaagtgcttcagtatctctgggcatgctctatatgcccaaggtttatattataatttttcatccagaacagaatgttcaaaaacgcaagaggagcttcaaggctgtggtgacagctgccaccatgcaaagcaaactgatccaaaaaggaaatgacagaccaaatggcgaggtgaaaagtgaactctgtgagagtcttgaaaccaacacttcctctaccaagacaacatatatcagttacagcaatcattcaatc

SEQ ID NO: 8 - protein, 908 aa, Homo sapiens
MVCEGKRSASCPCFFLLTAKFYWILTMMQRTHSQEYAHSIRVDGDIILGGLFPVHAKGERGVPCGELKKEKGIHRLEAMLYAIDQINKDPDLLSNITLGVRILDTCSRDTYALEQSLTFVQALIEKDASDVKCANGDPPIFTKPDKISGVIGAAASSVSIMVANILRLFKIPQISYASTAPELSDNTRYDFFSRVVPPDSYQAQAMVDIVTALGWNYVSTLASEGNYGESGVEAFTQISREIGGVCIAQSQKIPREPRPGEFEKIIKRLLETPNARAVIMFANEDDIRRILEAAKKLNQSGHFLWIGSDSWGSKIAPVYQQEEIAEGAVTILPKRASIDGFDRYFRSRTLANNRRNVWFAEFWEENFGCKLGSHGKRNSHIKKCTGLERIARDSSYEQEGKVQFVIDAVYSMAYALHNMHKDLCPGYIGLCPRMSTIDGKELLGYIRAVNFNGSAGTPVTFNENGDAPGRYDIFQYQITNKSTEYKVIGHWTNQLHLKVEDMQWAHREHTHPASVCSLPCKPGERKKTVKGVPCCWHCERCEGYNYQVDELSCELCPLDQRPNMNRTGCQLIPIIKLEWHSPWAVVPVFVAILGIIATTFVIVTFVRYNDTPIVRASGRELSYVLLTGIFLCYSITFLMIAAPDTIICSFRRVFLGLGMCFSYAALLTKTNRIHRIFEQGKKSVTAPKFISPASQLVITFSLISVQLLGVFVWFVVDPPHIIIDYGEQRTLDPEKARGVLKCDISDLSLICSLGYSILLMVTCTVYAIKTRGVPETFNEAKPIGFTMYTTCIIWLAFIPIFFGTAQSAEKMYIQTTTLTVSMSLSASVSLGMLYMPKVYIIIFHPEQNVQKRKRSFKAVVTAATMQSKLIQKGNDRPNGEVKSELCESLETNTSSTKTTYISYSNHSI

SEQ ID NO: 9 - protein, 228 aa, Homo sapiens
MPVKGGTKCIKYLLFGFNFIFWLAGIAVLAIGLWLRFDSQTKSIFEQETNNNNSSFYTGVYILIGAGALMMLVGFLGCCGAVQESQCMLGLFFGFLLVIFAIEIAAAIWGYSHKDEVIKEVQEFYKDTYNKLKTKDEPQRETLKAIHYALNCCGLAGGVEQFISDICPKKDVLETFTVKSCPDAIKEVFDNKFHIIGAVGIGIAVVMIFGMIFSMILCCAIRRNREMV

SEQ ID NO: 10 - DNA, 1246 bp, Homo sapiens
gaccagcctacagccgcctgcatctgtatccagcgccaggtcccgccagtcccagctgcgcgcgccccccagtcccgcacccgttcggcccaggctaagttagccctcaccatgccggtcaaaggaggcaccaagtgcatcaaatacctgctgttcggatttaacttcatcttctggcttgccgggattgctgtccttgccattggactatggctccgattcgactctcagaccaagagcatcttcgagcaagaaactaataataataattccagcttctacacaggagtctatattctgatcggagccggcgccctcatgatgctggtgggcttcctgggctgctgcggggctgtgcaggagtcccagtgcatgctgggactgttcttcggcttcctcttggtgatattcgccattgaaatagctgcggccatctggggatattcccacaaggatgaggtgattaaggaagtccaggagttttacaaggacacctacaacaagctgaaaaccaaggatgagccccagcgggaaacgctgaaagccatccactatgcgttgaactgctgtggtttggctgggggcgtggaacagtttatctcagacatctgccccaagaaggacgtactcgaaaccttcaccgtgaagtcctgtcctgatgccatcaaagaggtcttcgacaataaattccacatcatcggcgcagtgggcatcggcattgccgtggtcatgatatttggcatgatcttcagtatgatcttgtgctgtgctatccgcaggaaccgcgagatggtctagagtcagcttacatccctgagcaggaaagtttacccatgaagattggtgggattttttgtttgtttgttttgttttgtttgttgtttgttgtttgtttttttgccactaattttagtattcattctgcattgctagataaaagctgaagttactttatgtttgtcttttaatgcttcattcaatattgacatttgtagttgagcggggggtttggtttgctttggtttatattttttcagttgtttgtttttgcttgttatattaagcagaaatcctgcaatgaaaggtactatatttgctagactctagacaagatattgtacataaaagaatttttttgtctttaaatagatacaaatgtctatcaactttaatcaagttgtaacttatattgaagacaatttgatacataataaaaaattatgacaatgtcaaaaaaaaaaaaaaa

SEQ ID NO: 11 - protein, 238 aa, Homo sapiens
MAVEGGMKCVKFLLYVLLLAFCACAVGLIAVGVGAQLVLSQTIIQGATPGSLLPVVIIAVGVFLFLVAFVGCCGACKENYCLMITFAIFLSLIMLVEVAAAIAGYVFRDKVMSEFNNNFRQQMENYPKNNHTASILDRMQADFKCCGAANYTDWEKIPSMSKNRVPDSCCINVTVGCGINFNEKAIHKEGCVEKIGGWLRKNVLVVAAAALGIAFVEVLGIVFACCLVKSIRSGYEVM

SEQ ID NO: 12 - DNA, 714 bp, Homo sapiens
atggcggtggaaggaggaatgaaatgtgtgaagttcttgctctacgtcctcctgctggccttttgcgcctgtgcagtgggactgattgccgtgggtgtcggggcacagcttgtcctgagtcagaccataatccagggggctacccctggctctctgttgccagtggtcatcatcgcagtgggtgtcttcctcttcctggtggcttttgtgggctgctgcggggcctgcaaggagaactattgtcttatgatcacgtttgccatctttctgtctcttatcatgttggtggaggtggccgcagccattgctggctatgtgtttagagataaggtgatgtcagagtttaataacaacttccggcagcagatggagaattacccgaaaaacaaccacactgcttcgatcctggacaggatgcaggcagattttaagtgctgtggggctgctaactacacagattgggagaaaatcccttccatgtcgaagaaccgagtccccgactcctgctgcattaatgttactgtgggctgtgggattaatttcaacgagaaggcgatccataaggagggctgtgtggagaagattgggggctggctgaggaaaaatgtgctggtggtagctgcagcagcccttggaattgcttttgtcgaggttttgggaattgtctttgcctgctgcctcgtgaagagtatcagaagtggctacgaggtgatg

SEQ ID NO: 13 - protein, 236 aa, Homo sapiens
MGVEGCTKCIKYLLFVFNFVFWLAGGVILGVALWLRHDPQTTNLLYLELGDKPAPNTFYVGIYILIAVGAVMMFVGFLGCYGAIQESQCLLGTFFTCLVILFACEVAAGIWGFVNKDQIAKDVKQFYDQALQQAVVDDDANNAKAVVKTFHETLDCCGSSTLTALTTSVLKNNLCPSGSNIISNLFKEDCHQKIDDLFSGKLYLIGIAAIVVAVIMIFEMILSMVLCCGIRNSSVY

SEQ ID NO: 14 - DNA, 1482 bp, Homo sapiens
ggccagagagcgagcgcgcaacggcggcgacggcggcgaccccaccgcgcatcctgccaggcctccggcgcccagcgccccacgcgcccccgcgcccccgcgcccccgcgcccctttcttcgcgcccccgcccctcggcccgccaggcccccttgccggccacccgccaggccccgcgccggcccgcccgccgcccaggaccggcccgcgccccgcaggccgcccgccgcccgcgccgccatgggagtggagggctgcaccaagtgcatcaagtacctgctcttcgtcttcaatttcgtcttctggctggctggaggcgtgatcctgggtgtggccctgtggctccgccatgacccgcagaccaccaacctcctgtatctggagctgggagacaagcccgcgcccaacaccttctatgtaggcatctacatcctcatcgctgtgggcgctgtcatgatgttcgttggcttcctgggctgctacggggccatccaggaatcccagtgcctgctggggacgttcttcacctgcctggtcatcctgtttgcctgtgaggtggccgccggcatctggggctttgtcaacaaggaccagatcgccaaggatgtgaagcagttctatgaccaggccctacagcaggccgtggtggatgatgacgccaacaacgccaaggctgtggtgaagaccttccacgagacgcttgactgctgtggctccagcacactgactgctttgaccacctcagtgctcaagaacaatttgtgtccctcgggcagcaacatcatcagcaacctcttcaaggaggactgccaccagaagatcgatgacctcttctccgggaagctgtacctcatcggcattgctgccatcgtggtcgctgtgatcatgatcttcgagatgatcctgagcatggtgctgtgctgtggcatccggaacagctccgtgtactgaggccccgcagctctggccacagggacctctgcagtgccccctaagtgacccggacacttccgagggggccatcaccgcctgtgtatataacgtttccggtattactctgctacacgtagcctttttacttttggggttttgtttttgttctgaactttcctgttaccttttcagggctgacgtcacatgtaggtggcgtgtatgagtggagacgggcctgggtcttggggactggagggcaggggtccttctgccctggggtcccagggtgctctgcctgctcagccaggcctctcctgggagccactcgcccagagactcagcttggccaacttggggggctgtgtccacccagcccgcccgtcctgtgggctgcacagctcaccttgttccctcctgccccggttcgagagccgagtctgtgggcactctctgccttcatgcacctgtcctttctaacacgtcgccttcaactgtaatcacaacatcctgactccgtcatttaataaagaaggaacatcaggcatgcta